European Patent Specification EP 3 341 008 B1, published April 15, 2026. Title: PEPTIDES BINDING TO BFL-1. Applicant: DANA-FARBER CANCER INSTITUTE, INC. Application PCT/US2016/049095. The sequence listing filed with the application follows.

SEQUENCE LISTING (210 sequences)

SEQ ID NO: 1 - protein, 25 aa, Artificial Sequence
  Description of Artificial Sequence: Synthetic peptide
AELEVESATQLRRFGDKLNFRQKLL

SEQ ID NO: 2 - protein, 26 aa, Artificial Sequence
  Description of Artificial Sequence: Synthetic peptide
DMPREIWIAQELRRIGDEFNAYYARR

SEQ ID NO: 3 - protein, 27 aa, Artificial Sequence
  Description of Artificial Sequence: Synthetic peptide
QDASTKKLSESLKRIGDELDSNMELQR

SEQ ID NO: 4 - protein, 34 aa, Artificial Sequence
  Description of Artificial Sequence: Synthetic polypeptide
SSTMGQVGRQLAIIGDDINRRYDSEFQTMLQHLQ

SEQ ID NO: 5 - protein, 25 aa, Artificial Sequence
  Description of Artificial Sequence: Synthetic peptide
PGGRLAEVSTVLLRLGDELEQIRPS

SEQ ID NO: 6 - protein, 29 aa, Artificial Sequence
  Description of Artificial Sequence: Synthetic peptide
SESQEDIIRNIARHLAQVGDSMDRSIPPG

SEQ ID NO: 7 - protein, 33 aa, Artificial Sequence
  Description of Artificial Sequence: Synthetic polypeptide
EEEQWAREIGAQLRRMADDLNAQYERRRQEEQQ

SEQ ID NO: 8 - protein, 30 aa, Artificial Sequence
  Description of Artificial Sequence: Synthetic polypeptide
KKFEPKSGWMTFLEVTGKICEMLSLLKQYC

SEQ ID NO: 9 - protein, 25 aa, Artificial Sequence
  Description of Artificial Sequence: Synthetic peptide
  MOD_RES (13)..(13): Any non-natural amino acid
  MOD_RES (17)..(17): Any non-natural amino acid
AELEVECATQLRXFGDXLNFRQKLL

SEQ ID NO: 10 - protein, 25 aa, Artificial Sequence
  Description of Artificial Sequence: Synthetic peptide
  MOD_RES (13)..(13): Any non-natural amino acid
  MOD_RES (17)..(17): Any non-natural amino acid
AELEVECATQLRXFGDXLNFRQKDL

SEQ ID NO: 11 - protein, 25 aa, Artificial Sequence
  Description of Artificial Sequence: Synthetic peptide
  MOD_RES (13)..(13): Any non-natural amino acid
  MOD_RES (17)..(17): Any non-natural amino acid
AELEVELATQLRXFGDXLNFRQKLL

SEQ ID NO: 12 - protein, 25 aa, Artificial Sequence
  Description of Artificial Sequence: Synthetic peptide
  MOD_RES (13)..(13): Any non-natural amino acid
  MOD_RES (17)..(17): Any non-natural amino acid
AELEVECLTQLRXFGDXLNFRQKLL

SEQ ID NO: 13 - protein, 25 aa, Artificial Sequence
  Description of Artificial Sequence: Synthetic peptide
  MOD_RES (13)..(13): Any non-natural amino acid
  MOD_RES (17)..(17): Any non-natural amino acid
AELEVESATQLRXFGDXLNFRQKLL

SEQ ID NO: 14 - protein, 23 aa, Artificial Sequence
  Description of Artificial Sequence: Synthetic peptide
  MOD_RES (11)..(11): Any non-natural amino acid
  MOD_RES (15)..(15): Any non-natural amino acid
LEVECATQLRXFGDXLNFRQKLL

SEQ ID NO: 15 - protein, 22 aa, Artificial Sequence
  Description of Artificial Sequence: Synthetic peptide
  MOD_RES (13)..(13): Any non-natural amino acid
  MOD_RES (17)..(17): Any non-natural amino acid
AELEVECATQLRXFGDXLNFRQ

SEQ ID NO: 16 - protein, 25 aa, Artificial Sequence
  Description of Artificial Sequence: Synthetic peptide
  MOD_RES (13)..(13): Any non-natural amino acid
  MOD_RES (17)..(17): Any non-natural amino acid
AELEVECATQLRXYGDXLNFRQKLL

SEQ ID NO: 17 - protein, 25 aa, Artificial Sequence
  Description of Artificial Sequence: Synthetic peptide
  MOD_RES (13)..(13): Any non-natural amino acid
  MOD_RES (17)..(17): Any non-natural amino acid
AELEVECATQLRXIGDXLNFRQKLL

SEQ ID NO: 18 - protein, 20 aa, Artificial Sequence
  Description of Artificial Sequence: Synthetic peptide
  MOD_RES (9)..(9): Any non-natural amino acid
  MOD_RES (13)..(13): Any non-natural amino acid
VECATQLRXFGDXLNFRQKL

SEQ ID NO: 19 - protein, 20 aa, Artificial Sequence
  Description of Artificial Sequence: Synthetic peptide
  MOD_RES (9)..(9): Any non-natural amino acid
  MOD_RES (13)..(13): Any non-natural amino acid
VECATQLRXFGFXLNFRQKL

SEQ ID NO: 20 - protein, 25 aa, Artificial Sequence
  Description of Artificial Sequence: Synthetic peptide
  MOD_RES (6)..(6): Any non-natural amino acid
  MOD_RES (10)..(10): Any non-natural amino acid
AELEVXCATXLRRFGDKLNFRQKLL

SEQ ID NO: 21 - protein, 25 aa, Artificial Sequence
  Description of Artificial Sequence: Synthetic peptide
  MOD_RES (19)..(19): Any non-natural amino acid
  MOD_RES (23)..(23): Any non-natural amino acid
AELEVECATQLRRFGDKLXFRQXLL

SEQ ID NO: 22 - protein, 24 aa, Artificial Sequence
  Description of Artificial Sequence: Synthetic peptide
  MOD_RES (1)..(1): Non-natural electrophile containing amino acid or not present
  MOD_RES (11)..(11): Any non-natural amino acid
  MOD_RES (15)..(15): Any non-natural amino acid
XEVESATQLRXFGDXLNFRQKLLK

SEQ ID NO: 23 - protein, 20 aa, Artificial Sequence
  Description of Artificial Sequence: Synthetic peptide
  MOD_RES (1)..(1): Non-natural electrophile containing amino acid or not present
  MOD_RES (7)..(7): Any non-natural amino acid
  MOD_RES (11)..(11): Any non-natural amino acid
XATQLRXFGDXLNFRQKLLK

SEQ ID NO: 24 - protein, 23 aa, Artificial Sequence
  Description of Artificial Sequence: Synthetic peptide
  MOD_RES (1)..(1): Non-natural electrophile containing amino acid or not present
  MOD_RES (11)..(11): Any non-natural amino acid
  MOD_RES (15)..(15): Any non-natural amino acid
XEVESATQLRXFGDXLNFRQKLL

SEQ ID NO: 25 - protein, 19 aa, Artificial Sequence
  Description of Artificial Sequence: Synthetic peptide
  MOD_RES (1)..(1): Non-natural electrophile containing amino acid or not present
  MOD_RES (7)..(7): Any non-natural amino acid
  MOD_RES (11)..(11): Any non-natural amino acid
XATQLRXFGDXLNFRQKLL

SEQ ID NO: 26 - protein, 17 aa, Artificial Sequence
  Description of Artificial Sequence: Synthetic peptide
  MOD_RES (1)..(1): Non-natural electrophile containing amino acid or not present
  MOD_RES (8)..(8): Any non-natural amino acid
  MOD_RES (12)..(12): Any non-natural amino acid
XLSESLKXIGDXLDSNK

SEQ ID NO: 27 - protein, 19 aa, Artificial Sequence
  Description of Artificial Sequence: Synthetic peptide
  MOD_RES (1)..(1): Non-natural electrophile containing amino acid or not present
  MOD_RES (7)..(7): Any non-natural amino acid
  MOD_RES (11)..(11): Any non-natural amino acid
XAQELRXIGDXFNAYYARK

SEQ ID NO: 28 - protein, 20 aa, Artificial Sequence
  Description of Artificial Sequence: Synthetic peptide
  MOD_RES (1)..(1): Non-natural electrophile containing amino acid or not present
  MOD_RES (8)..(8): Any non-natural amino acid
  MOD_RES (12)..(12): Any non-natural amino acid
XIAQELRXIGDXFNAYYARK

SEQ ID NO: 29 - protein, 19 aa, Artificial Sequence
  Description of Artificial Sequence: Synthetic peptide
  MOD_RES (1)..(1): Non-natural electrophile containing amino acid or not present
  MOD_RES (7)..(7): Any non-natural amino acid
  MOD_RES (11)..(11): Any non-natural amino acid
XAQELRXIGDXFNAYYARR

SEQ ID NO: 30 - protein, 20 aa, Artificial Sequence
  Description of Artificial Sequence: Synthetic peptide
  MOD_RES (1)..(1): Non-natural electrophile containing amino acid or not present
  MOD_RES (8)..(8): Any non-natural amino acid
  MOD_RES (12)..(12): Any non-natural amino acid
XIAQELRXIGDXFNAYYARR

SEQ ID NO: 31 - protein, 16 aa, Artificial Sequence
  Description of Artificial Sequence: Synthetic peptide
  MOD_RES (1)..(1): Non-natural electrophile containing amino acid or not present
  MOD_RES (4)..(4): Any non-natural amino acid
  MOD_RES (8)..(8): Any non-natural amino acid
XVGXQLAXIGDDINRR

SEQ ID NO: 32 - protein, 15 aa, Artificial Sequence
  Description of Artificial Sequence: Synthetic peptide
  MOD_RES (1)..(1): Non-natural electrophile containing amino acid or not present
  MOD_RES (3)..(3): Any non-natural amino acid
  MOD_RES (7)..(7): Any non-natural amino acid
  MOD_RES (15)..(15): May or may not be present
XGXQLAXIGDDINRR

SEQ ID NO: 33 - protein, 16 aa, Artificial Sequence
  Description of Artificial Sequence: Synthetic peptide
  MOD_RES (1)..(1): Non-natural electrophile containing amino acid or not present
XEVSTVLLRLGDELEQ

SEQ ID NO: 34 - protein, 15 aa, Artificial Sequence
  Description of Artificial Sequence: Synthetic peptide
  MOD_RES (1)..(1): Non-natural electrophile containing amino acid or not present
XVSTVLLRLGDELEQ

SEQ ID NO: 35 - protein, 14 aa, Artificial Sequence
  Description of Artificial Sequence: Synthetic peptide
  MOD_RES (1)..(1): Non-natural electrophile containing amino acid or not present
XSTVLLRLGDELEQ

SEQ ID NO: 36 - protein, 13 aa, Artificial Sequence
  Description of Artificial Sequence: Synthetic peptide
  MOD_RES (1)..(1): Non-natural electrophile containing amino acid or not present
XTVLLRLGDELEQ

SEQ ID NO: 37 - protein, 16 aa, Artificial Sequence
  Description of Artificial Sequence: Synthetic peptide
GQVGRQLAIIGDDINR

SEQ ID NO: 38 - protein, 21 aa, Artificial Sequence
  Description of Artificial Sequence: Synthetic peptide
IWIAQELRRIGDEFNAYYARR

SEQ ID NO: 39 - protein, 16 aa, Artificial Sequence
  Description of Artificial Sequence: Synthetic peptide
KLSECLKRIGDELDSN

SEQ ID NO: 40 - protein, 16 aa, Artificial Sequence
  Description of Artificial Sequence: Synthetic peptide
LAECTVLLRLGDELEQ

SEQ ID NO: 41 - protein, 22 aa, Artificial Sequence
  Description of Artificial Sequence: Synthetic peptide
  MOD_RES (1)..(1): Non-natural electrophile containing amino acid or not present
XDIIRNIARHLAQVGDSMDRSI

SEQ ID NO: 42 - protein, 22 aa, Artificial Sequence
  Description of Artificial Sequence: Synthetic peptide
  MOD_RES (3)..(3): Non-natural electrophile containing amino acid or not present
EDXIRNIARHLAQVGDSMDRSI

SEQ ID NO: 43 - protein, 22 aa, Artificial Sequence
  Description of Artificial Sequence: Synthetic peptide
  MOD_RES (6)..(6): Non-natural electrophile containing amino acid or not present
EDIIRXIARHLAQVGDSMDRSI

SEQ ID NO: 44 - protein, 22 aa, Artificial Sequence
  Description of Artificial Sequence: Synthetic peptide
  MOD_RES (7)..(7): Non-natural electrophile containing amino acid or not present
EDIIRNXARHLAQVGDSMDRSI

SEQ ID NO: 45 - protein, 19 aa, Artificial Sequence
  Description of Artificial Sequence: Synthetic peptide
  MOD_RES (1)..(1): Non-natural electrophile containing amino acid or not present
  MOD_RES (12)..(12): Any non-natural amino acid
  MOD_RES (16)..(16): Any non-natural amino acid
  MOD_RES (17)..(17): Norleucine
XIIRNIARHLAXVGDXXDR

SEQ ID NO: 46 - protein, 18 aa, Artificial Sequence
  Description of Artificial Sequence: Synthetic peptide
  MOD_RES (1)..(1): Non-natural electrophile containing amino acid or not present
  MOD_RES (11)..(11): Any non-natural amino acid
  MOD_RES (15)..(15): Any non-natural amino acid
  MOD_RES (16)..(16): Norleucine
XIRNIARHLAXVGDXXDR

SEQ ID NO: 47 - protein, 15 aa, Artificial Sequence
  Description of Artificial Sequence: Synthetic peptide
  MOD_RES (1)..(1): Non-natural electrophile containing amino acid or not present
  MOD_RES (8)..(8): Any non-natural amino acid
  MOD_RES (12)..(12): Any non-natural amino acid
  MOD_RES (13)..(13): Norleucine
XIARHLAXVGDXXDR

SEQ ID NO: 48 - protein, 14 aa, Artificial Sequence
  Description of Artificial Sequence: Synthetic peptide
  MOD_RES (1)..(1): Non-natural electrophile containing amino acid or not present
  MOD_RES (7)..(7): Any non-natural amino acid
  MOD_RES (11)..(11): Any non-natural amino acid
  MOD_RES (12)..(12): Norleucine
XARHLAXVGDXXDR

SEQ ID NO: 49 - protein, 16 aa, Artificial Sequence
  Description of Artificial Sequence: Synthetic peptide
  MOD_RES (1)..(1): Non-natural electrophile containing amino acid or not present
  MOD_RES (2)..(2): Any non-natural amino acid
  MOD_RES (6)..(6): Any non-natural amino acid
XXTQLXRFGDKLNFRQ

SEQ ID NO: 50 - protein, 16 aa, Artificial Sequence
  Description of Artificial Sequence: Synthetic peptide
  MOD_RES (1)..(1): Non-natural electrophile containing amino acid or not present
  MOD_RES (3)..(3): Any non-natural amino acid
  MOD_RES (7)..(7): Any non-natural amino acid
XAXQLRXFGDKLNFRQ

SEQ ID NO: 51 - protein, 16 aa, Artificial Sequence
  Description of Artificial Sequence: Synthetic peptide
  MOD_RES (1)..(1): Non-natural electrophile containing amino acid or not present
  MOD_RES (4)..(4): Any non-natural amino acid
  MOD_RES (8)..(8): Any non-natural amino acid
XATXLRRXGDKLNFRQ

SEQ ID NO: 52 - protein, 16 aa, Artificial Sequence
  Description of Artificial Sequence: Synthetic peptide
  MOD_RES (1)..(1): Non-natural electrophile containing amino acid or not present
  MOD_RES (5)..(5): Any non-natural amino acid
  MOD_RES (9)..(9): Any non-natural amino acid
XATQXRRFXDKLNFRQ

SEQ ID NO: 53 - protein, 16 aa, Artificial Sequence
  Description of Artificial Sequence: Synthetic peptide
  MOD_RES (1)..(1): Non-natural electrophile containing amino acid or not present
  MOD_RES (6)..(6): Any non-natural amino acid
  MOD_RES (10)..(10): Any non-natural amino acid
XATQLXRFGXKLNFRQ

SEQ ID NO: 54 - protein, 16 aa, Artificial Sequence
  Description of Artificial Sequence: Synthetic peptide
  MOD_RES (1)..(1): Non-natural electrophile containing amino acid or not present
  MOD_RES (7)..(7): Any non-natural amino acid
  MOD_RES (11)..(11): Any non-natural amino acid
XATQLRXFGDXLNFRQ

SEQ ID NO: 55 - protein, 16 aa, Artificial Sequence
  Description of Artificial Sequence: Synthetic peptide
  MOD_RES (1)..(1): Non-natural electrophile containing amino acid or not present
  MOD_RES (8)..(8): Any non-natural amino acid
  MOD_RES (12)..(12): Any non-natural amino acid
XATQLRRXGDKXNFRQ

SEQ ID NO: 56 - protein, 16 aa, Artificial Sequence
  Description of Artificial Sequence: Synthetic peptide
  MOD_RES (1)..(1): Non-natural electrophile containing amino acid or not present
  MOD_RES (9)..(9): Any non-natural amino acid
  MOD_RES (13)..(13): Any non-natural amino acid
XATQLRRFXDKLXFRQ

SEQ ID NO: 57 - protein, 16 aa, Artificial Sequence
  Description of Artificial Sequence: Synthetic peptide
  MOD_RES (1)..(1): Non-natural electrophile containing amino acid or not present
  MOD_RES (10)..(10): Any non-natural amino acid
  MOD_RES (14)..(14): Any non-natural amino acid
XATQLRRFGXKLNXRQ

SEQ ID NO: 58 - protein, 16 aa, Artificial Sequence
  Description of Artificial Sequence: Synthetic peptide
  MOD_RES (1)..(1): Non-natural electrophile containing amino acid or not present
  MOD_RES (12)..(12): Any non-natural amino acid
  MOD_RES (16)..(16): Any non-natural amino acid
XATQLRRFGDKXNFRX

SEQ ID NO: 59 - protein, 17 aa, Artificial Sequence
  Description of Artificial Sequence: Synthetic peptide
  MOD_RES (1)..(1): Non-natural electrophile containing amino acid or not present
  MOD_RES (13)..(13): Any non-natural amino acid
  MOD_RES (17)..(17): Any non-natural amino acid
XATQLRRFGDKLXFRQX

SEQ ID NO: 60 - protein, 16 aa, Artificial Sequence
  Description of Artificial Sequence: Synthetic peptide
  MOD_RES (1)..(1): Non-natural electrophile containing amino acid or not present
  MOD_RES (2)..(2): R-octenyl alanine
  MOD_RES (9)..(9): Any non-natural amino acid
XATQLRRFXDKLNFRQ

SEQ ID NO: 61 - protein, 16 aa, Artificial Sequence
  Description of Artificial Sequence: Synthetic peptide
  MOD_RES (1)..(1): Non-natural electrophile containing amino acid or not present
  MOD_RES (3)..(3): R-octenyl alanine
  MOD_RES (10)..(10): Any non-natural amino acid
XAAQLRRFGXKLNFRQ

SEQ ID NO: 62 - protein, 16 aa, Artificial Sequence
  Description of Artificial Sequence: Synthetic peptide
  MOD_RES (1)..(1): Non-natural electrophile containing amino acid or not present
  MOD_RES (4)..(4): R-octenyl alanine
  MOD_RES (11)..(11): Any non-natural amino acid
XATALRRFGDXLNFRQ

SEQ ID NO: 63 - protein, 16 aa, Artificial Sequence
  Description of Artificial Sequence: Synthetic peptide
  MOD_RES (1)..(1): Non-natural electrophile containing amino acid or not present
  MOD_RES (5)..(5): R-octenyl alanine
  MOD_RES (12)..(12): Any non-natural amino acid
XATQARRFGDKXNFRQ

SEQ ID NO: 64 - protein, 16 aa, Artificial Sequence
  Description of Artificial Sequence: Synthetic peptide
  MOD_RES (1)..(1): Non-natural electrophile containing amino acid or not present
  MOD_RES (6)..(6): R-octenyl alanine
  MOD_RES (13)..(13): Any non-natural amino acid
XATQLARFGDKLXFRQ

SEQ ID NO: 65 - protein, 16 aa, Artificial Sequence
  Description of Artificial Sequence: Synthetic peptide
  MOD_RES (1)..(1): Non-natural electrophile containing amino acid or not present
  MOD_RES (7)..(7): R-octenyl alanine
  MOD_RES (14)..(14): Any non-natural amino acid
XATQLRAFGDKLNXRQ

SEQ ID NO: 66 - protein, 16 aa, Artificial Sequence
  Description of Artificial Sequence: Synthetic peptide
  MOD_RES (1)..(1): Non-natural electrophile containing amino acid or not present
  MOD_RES (8)..(8): R-octenyl alanine
  MOD_RES (15)..(15): Any non-natural amino acid
XATQLRRAGDKLNFXQ

SEQ ID NO: 67 - protein, 16 aa, Artificial Sequence
  Description of Artificial Sequence: Synthetic peptide
  MOD_RES (1)..(1): Non-natural electrophile containing amino acid or not present
  MOD_RES (9)..(9): R-octenyl alanine
  MOD_RES (16)..(16): Any non-natural amino acid
XATQLRRFADKLNFRX

SEQ ID NO: 68 - protein, 14 aa, Artificial Sequence
  Description of Artificial Sequence: Synthetic peptide
  MOD_RES (1)..(1): Non-natural electrophile containing amino acid or not present
  MOD_RES (2)..(2): Any non-natural amino acid
  MOD_RES (6)..(6): Any non-natural amino acid
XXRQLXIIGDDINR

SEQ ID NO: 69 - protein, 14 aa, Artificial Sequence
  Description of Artificial Sequence: Synthetic peptide
  MOD_RES (1)..(1): Non-natural electrophile containing amino acid or not present
  MOD_RES (4)..(4): Any non-natural amino acid
  MOD_RES (8)..(8): Any non-natural amino acid
XGRXLAIXGDDINR

SEQ ID NO: 70 - protein, 14 aa, Artificial Sequence
  Description of Artificial Sequence: Synthetic peptide
  MOD_RES (1)..(1): Non-natural electrophile containing amino acid or not present
  MOD_RES (5)..(5): Any non-natural amino acid
  MOD_RES (9)..(9): Any non-natural amino acid
XGRQXAIIXDDINR

SEQ ID NO: 71 - protein, 14 aa, Artificial Sequence
  Description of Artificial Sequence: Synthetic peptide
  MOD_RES (1)..(1): Non-natural electrophile containing amino acid or not present
  MOD_RES (6)..(6): Any non-natural amino acid
  MOD_RES (10)..(10): Any non-natural amino acid
XGRQLXIIGXDINR

SEQ ID NO: 72 - protein, 14 aa, Artificial Sequence
  Description of Artificial Sequence: Synthetic peptide
  MOD_RES (1)..(1): Non-natural electrophile containing amino acid or not present
  MOD_RES (7)..(7): Any non-natural amino acid
  MOD_RES (11)..(11): Any non-natural amino acid
XGRQLAXIGDXINR

SEQ ID NO: 73 - protein, 14 aa, Artificial Sequence
  Description of Artificial Sequence: Synthetic peptide
  MOD_RES (1)..(1): Non-natural electrophile containing amino acid or not present
  MOD_RES (8)..(8): Any non-natural amino acid
  MOD_RES (12)..(12): Any non-natural amino acid
XGRQLAIXGDDXNR

SEQ ID NO: 74 - protein, 14 aa, Artificial Sequence
  Description of Artificial Sequence: Synthetic peptide
  MOD_RES (1)..(1): Non-natural electrophile containing amino acid or not present
  MOD_RES (9)..(9): Any non-natural amino acid
  MOD_RES (13)..(13): Any non-natural amino acid
XGRQLAIIXDDIXR

SEQ ID NO: 75 - protein, 14 aa, Artificial Sequence
  Description of Artificial Sequence: Synthetic peptide
  MOD_RES (1)..(1): Non-natural electrophile containing amino acid or not present
  MOD_RES (10)..(10): Any non-natural amino acid
  MOD_RES (14)..(14): Any non-natural amino acid
XGRQLAIIGXDINX

SEQ ID NO: 76 - protein, 15 aa, Artificial Sequence
  Description of Artificial Sequence: Synthetic peptide
  MOD_RES (1)..(1): Non-natural electrophile containing amino acid or not present
  MOD_RES (11)..(11): Any non-natural amino acid
  MOD_RES (15)..(15): Any non-natural amino acid
XGRQLAIIGDXINRX

SEQ ID NO: 77 - protein, 14 aa, Artificial Sequence
  Description of Artificial Sequence: Synthetic peptide
  MOD_RES (1)..(1): Non-natural electrophile containing amino acid or not present
  MOD_RES (2)..(2): R-octenyl alanine
  MOD_RES (9)..(9): Any non-natural amino acid
XARQLAIIXDDINR

SEQ ID NO: 78 - protein, 14 aa, Artificial Sequence
  Description of Artificial Sequence: Synthetic peptide
  MOD_RES (1)..(1): Non-natural electrophile containing amino acid or not present
  MOD_RES (3)..(3): R-octenyl alanine
  MOD_RES (10)..(10): Any non-natural amino acid
XGAQLAIIGXDINR

SEQ ID NO: 79 - protein, 14 aa, Artificial Sequence
  Description of Artificial Sequence: Synthetic peptide
  MOD_RES (1)..(1): Non-natural electrophile containing amino acid or not present
  MOD_RES (4)..(4): R-octenyl alanine
  MOD_RES (11)..(11): Any non-natural amino acid
XGRALAIIGDXINR

SEQ ID NO: 80 - protein, 14 aa, Artificial Sequence
  Description of Artificial Sequence: Synthetic peptide
  MOD_RES (1)..(1): Non-natural electrophile containing amino acid or not present
  MOD_RES (5)..(5): R-octenyl alanine
  MOD_RES (12)..(12): Any non-natural amino acid
XGRQAAIIGDDXNR

SEQ ID NO: 81 - protein, 14 aa, Artificial Sequence
  Description of Artificial Sequence: Synthetic peptide
  MOD_RES (1)..(1): Non-natural electrophile containing amino acid or not present
  MOD_RES (6)..(6): R-octenyl alanine
  MOD_RES (13)..(13): Any non-natural amino acid
XGRQLAIIGDDIXR

SEQ ID NO: 82 - protein, 14 aa, Artificial Sequence
  Description of Artificial Sequence: Synthetic peptide
  MOD_RES (1)..(1): Non-natural electrophile containing amino acid or not present
  MOD_RES (7)..(7): R-octenyl alanine
  MOD_RES (14)..(14): Any non-natural amino acid
XGRQLAAIGDDINX

SEQ ID NO: 83 - protein, 15 aa, Artificial Sequence
  Description of Artificial Sequence: Synthetic peptide
  MOD_RES (1)..(1): Non-natural electrophile containing amino acid or not present
  MOD_RES (8)..(8): R-octenyl alanine
  MOD_RES (15)..(15): Any non-natural amino acid
XGRQLAIAGDDINRX

SEQ ID NO: 84 - protein, 15 aa, Artificial Sequence
  Description of Artificial Sequence: Synthetic peptide
  MOD_RES (1)..(1): Non-natural electrophile containing amino acid or not present
  MOD_RES (3)..(3): Any non-natural amino acid
  MOD_RES (7)..(7): Any non-natural amino acid
XVXRQLXIIGDDINR

SEQ ID NO: 85 - protein, 15 aa, Artificial Sequence
  Description of Artificial Sequence: Synthetic peptide
  MOD_RES (1)..(1): Non-natural electrophile containing amino acid or not present
  MOD_RES (4)..(4): Any non-natural amino acid
  MOD_RES (8)..(8): Any non-natural amino acid
XVGXQLAXIGDDINR

SEQ ID NO: 86 - protein, 15 aa, Artificial Sequence
  Description of Artificial Sequence: Synthetic peptide
  MOD_RES (1)..(1): Non-natural electrophile containing amino acid or not present
  MOD_RES (5)..(5): Any non-natural amino acid
  MOD_RES (9)..(9): Any non-natural amino acid
XVGRXLAIXGDDINR

SEQ ID NO: 87 - protein, 15 aa, Artificial Sequence
  Description of Artificial Sequence: Synthetic peptide
  MOD_RES (1)..(1): Non-natural electrophile containing amino acid or not present
  MOD_RES (6)..(6): Any non-natural amino acid
  MOD_RES (10)..(10): Any non-natural amino acid
XVGRQXAIIXDDINR

SEQ ID NO: 88 - protein, 15 aa, Artificial Sequence
  Description of Artificial Sequence: Synthetic peptide
  MOD_RES (1)..(1): Non-natural electrophile containing amino acid or not present
  MOD_RES (7)..(7): Any non-natural amino acid
  MOD_RES (11)..(11): Any non-natural amino acid
XVGRQLXIIGXDINR

SEQ ID NO: 89 - protein, 15 aa, Artificial Sequence
  Description of Artificial Sequence: Synthetic peptide
  MOD_RES (1)..(1): Non-natural electrophile containing amino acid or not present
  MOD_RES (8)..(8): Any non-natural amino acid
  MOD_RES (12)..(12): Any non-natural amino acid
XVGRQLAXIGDXINR

SEQ ID NO: 90 - protein, 15 aa, Artificial Sequence
  Description of Artificial Sequence: Synthetic peptide
  MOD_RES (1)..(1): Non-natural electrophile containing amino acid or not present
  MOD_RES (9)..(9): Any non-natural amino acid
  MOD_RES (13)..(13): Any non-natural amino acid
XVGRQLAIXGDDXNR

SEQ ID NO: 91 - protein, 15 aa, Artificial Sequence
  Description of Artificial Sequence: Synthetic peptide
  MOD_RES (1)..(1): Non-natural electrophile containing amino acid or not present
  MOD_RES (10)..(10): Any non-natural amino acid
  MOD_RES (14)..(14): Any non-natural amino acid
XVGRQLAIIXDDIXR

SEQ ID NO: 92 - protein, 15 aa, Artificial Sequence
  Description of Artificial Sequence: Synthetic peptide
  MOD_RES (1)..(1): Non-natural electrophile containing amino acid or not present
  MOD_RES (11)..(11): Any non-natural amino acid
  MOD_RES (15)..(15): Any non-natural amino acid
XVGRQLAIIGXDINX

SEQ ID NO: 93 - protein, 16 aa, Artificial Sequence
  Description of Artificial Sequence: Synthetic peptide
  MOD_RES (1)..(1): Non-natural electrophile containing amino acid or not present
  MOD_RES (12)..(12): Any non-natural amino acid
  MOD_RES (16)..(16): Any non-natural amino acid
XVGRQLAIIGDXINRX

SEQ ID NO: 94 - protein, 15 aa, Artificial Sequence
  Description of Artificial Sequence: Synthetic peptide
  MOD_RES (1)..(1): Non-natural electrophile containing amino acid or not present
  MOD_RES (3)..(3): R-octenyl alanine
  MOD_RES (10)..(10): Any non-natural amino acid
XVARQLAIIXDDINR

SEQ ID NO: 95 - protein, 15 aa, Artificial Sequence
  Description of Artificial Sequence: Synthetic peptide
  MOD_RES (1)..(1): Non-natural electrophile containing amino acid or not present
  MOD_RES (4)..(4): R-octenyl alanine
  MOD_RES (11)..(11): Any non-natural amino acid
XVGAQLAIIGXDINR

SEQ ID NO: 96 - protein, 15 aa, Artificial Sequence
  Description of Artificial Sequence: Synthetic peptide
  MOD_RES (1)..(1): Non-natural electrophile containing amino acid or not present
  MOD_RES (5)..(5): R-octenyl alanine
  MOD_RES (12)..(12): Any non-natural amino acid
XVGRALAIIGDXINR

SEQ ID NO: 97 - protein, 15 aa, Artificial Sequence
  Description of Artificial Sequence: Synthetic peptide
  MOD_RES (1)..(1): Non-natural electrophile containing amino acid or not present
  MOD_RES (6)..(6): R-octenyl alanine
  MOD_RES (13)..(13): Any non-natural amino acid
XVGRQAAIIGDDXNR

SEQ ID NO: 98 - protein, 15 aa, Artificial Sequence
  Description of Artificial Sequence: Synthetic peptide
  MOD_RES (1)..(1): Non-natural electrophile containing amino acid or not present
  MOD_RES (7)..(7): R-octenyl alanine
  MOD_RES (14)..(14): Any non-natural amino acid
XVGRQLAIIGDDIXR

SEQ ID NO: 99 - protein, 15 aa, Artificial Sequence
  Description of Artificial Sequence: Synthetic peptide
  MOD_RES (1)..(1): Non-natural electrophile containing amino acid or not present
  MOD_RES (8)..(8): R-octenyl alanine
  MOD_RES (15)..(15): Any non-natural amino acid
XVGRQLAAIGDDINX

SEQ ID NO: 100 - protein, 16 aa, Artificial Sequence
  Description of Artificial Sequence: Synthetic peptide
  MOD_RES (1)..(1): Non-natural electrophile containing amino acid or not present
  MOD_RES (9)..(9): R-octenyl alanine
  MOD_RES (16)..(16): Any non-natural amino acid
XVGRQLAIAGDDINRX

SEQ ID NO: 101 - protein, 15 aa, Artificial Sequence
  Description of Artificial Sequence: Synthetic peptide
  MOD_RES (1)..(1): Non-natural electrophile containing amino acid or not present
  MOD_RES (2)..(2): Any non-natural amino acid
  MOD_RES (6)..(6): Any non-natural amino acid
XXSESXKRIGDELDS

SEQ ID NO: 102 - protein, 15 aa, Artificial Sequence
  Description of Artificial Sequence: Synthetic peptide
  MOD_RES (1)..(1): Non-natural electrophile containing amino acid or not present
  MOD_RES (3)..(3): Any non-natural amino acid
  MOD_RES (7)..(7): Any non-natural amino acid
XLXESLXRIGDELDS

SEQ ID NO: 103 - protein, 15 aa, Artificial Sequence
  Description of Artificial Sequence: Synthetic peptide
  MOD_RES (1)..(1): Non-natural electrophile containing amino acid or not present
  MOD_RES (4)..(4): Any non-natural amino acid
  MOD_RES (8)..(8): Any non-natural amino acid
XLSXSLKXIGDELDS

SEQ ID NO: 104 - protein, 15 aa, Artificial Sequence
  Description of Artificial Sequence: Synthetic peptide
  MOD_RES (1)..(1): Non-natural electrophile containing amino acid or not present
  MOD_RES (5)..(5): Any non-natural amino acid
  MOD_RES (9)..(9): Any non-natural amino acid
XLSEXLKRXGDELDS

SEQ ID NO: 105 - protein, 15 aa, Artificial Sequence
  Description of Artificial Sequence: Synthetic peptide
  MOD_RES (1)..(1): Non-natural electrophile containing amino acid or not present
  MOD_RES (6)..(6): Any non-natural amino acid
  MOD_RES (10)..(10): Any non-natural amino acid
XLSESXKRIXDELDS

SEQ ID NO: 106 - protein, 15 aa, Artificial Sequence
  Description of Artificial Sequence: Synthetic peptide
  MOD_RES (1)..(1): Non-natural electrophile containing amino acid or not present
  MOD_RES (7)..(7): Any non-natural amino acid
  MOD_RES (11)..(11): Any non-natural amino acid
XLSESLXRIGXELDS

SEQ ID NO: 107 - protein, 15 aa, Artificial Sequence
  Description of Artificial Sequence: Synthetic peptide
  MOD_RES (1)..(1): Non-natural electrophile containing amino acid or not present
  MOD_RES (8)..(8): Any non-natural amino acid
  MOD_RES (12)..(12): Any non-natural amino acid
XLSESLKXIGDXLDS

SEQ ID NO: 108 - protein, 15 aa, Artificial Sequence
  Description of Artificial Sequence: Synthetic peptide
  MOD_RES (1)..(1): Non-natural electrophile containing amino acid or not present
  MOD_RES (9)..(9): Any non-natural amino acid
  MOD_RES (13)..(13): Any non-natural amino acid
XLSESLKRXGDEXDS

SEQ ID NO: 109 - protein, 15 aa, Artificial Sequence
  Description of Artificial Sequence: Synthetic peptide
  MOD_RES (1)..(1): Non-natural electrophile containing amino acid or not present
  MOD_RES (10)..(10): Any non-natural amino acid
  MOD_RES (14)..(14): Any non-natural amino acid
XLSESLKRIXDELXS

SEQ ID NO: 110 - protein, 15 aa, Artificial Sequence
  Description of Artificial Sequence: Synthetic peptide
  MOD_RES (1)..(1): Non-natural electrophile containing amino acid or not present
  MOD_RES (11)..(11): Any non-natural amino acid
  MOD_RES (15)..(15): Any non-natural amino acid
XLSESLKRIGXELDX

SEQ ID NO: 111 - protein, 16 aa, Artificial Sequence
  Description of Artificial Sequence: Synthetic peptide
  MOD_RES (1)..(1): Non-natural electrophile containing amino acid or not present
  MOD_RES (12)..(12): Any non-natural amino acid
  MOD_RES (16)..(16): Any non-natural amino acid
XLSESLKRIGDXLDSX

SEQ ID NO: 112 - protein, 15 aa, Artificial Sequence
  Description of Artificial Sequence: Synthetic peptide
  MOD_RES (1)..(1): Non-natural electrophile containing amino acid or not present
  MOD_RES (2)..(2): R-octenyl alanine
  MOD_RES (9)..(9): Any non-natural amino acid
XASESLKRXGDELDS

SEQ ID NO: 113 - protein, 15 aa, Artificial Sequence
  Description of Artificial Sequence: Synthetic peptide
  MOD_RES (1)..(1): Non-natural electrophile containing amino acid or not present
  MOD_RES (3)..(3): R-octenyl alanine
  MOD_RES (10)..(10): Any non-natural amino acid
XLAESLKRIXDELDS

SEQ ID NO: 114 - protein, 15 aa, Artificial Sequence
  Description of Artificial Sequence: Synthetic peptide
  MOD_RES (1)..(1): Non-natural electrophile containing amino acid or not present
  MOD_RES (4)..(4): R-octenyl alanine
  MOD_RES (11)..(11): Any non-natural amino acid
XLSASLKRIGXELDS

SEQ ID NO: 115 - protein, 15 aa, Artificial Sequence
  Description of Artificial Sequence: Synthetic peptide
  MOD_RES (1)..(1): Non-natural electrophile containing amino acid or not present
  MOD_RES (5)..(5): R-octenyl alanine
  MOD_RES (12)..(12): Any non-natural amino acid
XLSEALKRIGDXLDS

SEQ ID NO: 116 - protein, 15 aa, Artificial Sequence
  Description of Artificial Sequence: Synthetic peptide
  MOD_RES (1)..(1): Non-natural electrophile containing amino acid or not present
  MOD_RES (6)..(6): R-octenyl alanine
  MOD_RES (13)..(13): Any non-natural amino acid
XLSESAKRIGDEXDS

SEQ ID NO: 117 - protein, 15 aa, Artificial Sequence
  Description of Artificial Sequence: Synthetic peptide
  MOD_RES (1)..(1): Non-natural electrophile containing amino acid or not present
  MOD_RES (7)..(7): R-octenyl alanine
  MOD_RES (14)..(14): Any non-natural amino acid
XLSESLARIGDELXS

SEQ ID NO: 118 - protein, 15 aa, Artificial Sequence
  Description of Artificial Sequence: Synthetic peptide
  MOD_RES (1)..(1): Non-natural electrophile containing amino acid or not present
  MOD_RES (8)..(8): R-octenyl alanine
  MOD_RES (15)..(15): Any non-natural amino acid
XLSESLKAIGDELDX

SEQ ID NO: 119 - protein, 16 aa, Artificial Sequence
  Description of Artificial Sequence: Synthetic peptide
  MOD_RES (1)..(1): Non-natural electrophile containing amino acid or not present
  MOD_RES (9)..(9): R-octenyl alanine
  MOD_RES (16)..(16): Any non-natural amino acid
XLSESLKRAGDELDSX

SEQ ID NO: 120 - skipped

SEQ ID NO: 121 - protein, 15 aa, Artificial Sequence
  Description of Artificial Sequence: Synthetic peptide
ATQLRRFGDKLNFRQ

SEQ ID NO: 122 - protein, 26 aa, Artificial Sequence
  Description of Artificial Sequence: Synthetic peptide
AELEVECATQLRRFGDKLNFRQKLLN

SEQ ID NO: 123 - protein, 22 aa, Artificial Sequence
  Description of Artificial Sequence: Synthetic peptide
EIWIAQELRRIGDEFNAYYARR

SEQ ID NO: 124 - protein, 21 aa, Artificial Sequence
  Description of Artificial Sequence: Synthetic peptide
DIIRNIARHLAQVGDSMDRSI

SEQ ID NO: 125 - protein, 22 aa, Artificial Sequence
  Description of Artificial Sequence: Synthetic peptide
SSTMGQVGRQLAIIGDDINRRY

SEQ ID NO: 126 - protein, 25 aa, Artificial Sequence
  Description of Artificial Sequence: Synthetic peptide
QDASTKKLSESLKRIGDELDSNMEL

SEQ ID NO: 127 - protein, 20 aa, Artificial Sequence
  Description of Artificial Sequence: Synthetic peptide
RLAEVCAVLLRLGDELEMIR

SEQ ID NO: 128 - protein, 19 aa, Artificial Sequence
  Description of Artificial Sequence: Synthetic peptide
  MOD_RES (1)..(1): Non-natural electrophile containing amino acid or not present
XATQLRRFGDKLNFRQKLL

SEQ ID NO: 129 - protein, 23 aa, Artificial Sequence
  Description of Artificial Sequence: Synthetic peptide
  MOD_RES (1)..(1): Non-natural electrophile containing amino acid or not present
XEVESATQLRRFGDKLNFRQKLL

SEQ ID NO: 130 - protein, 20 aa, Artificial Sequence
  Description of Artificial Sequence: Synthetic peptide
  MOD_RES (1)..(1): Non-natural electrophile containing amino acid or not present
XIAQELRRIGDEFNAYYARR

SEQ ID NO: 131 - protein, 15 aa, Artificial Sequence
  Description of Artificial Sequence: Synthetic peptide
ATQLRRFGDKLNFRQ

SEQ ID NO: 132 - protein, 19 aa, Artificial Sequence
  Description of Artificial Sequence: Synthetic peptide
IAQELRRIGDEFNAYYARR

SEQ ID NO: 133 - protein, 13 aa, Artificial Sequence
  Description of Artificial Sequence: Synthetic peptide
ARHLAQVGDSMDR

SEQ ID NO: 134 - protein, 13 aa, Artificial Sequence
  Description of Artificial Sequence: Synthetic peptide
GRQLAIIGDDINR

SEQ ID NO: 135 - protein, 14 aa, Artificial Sequence
  Description of Artificial Sequence: Synthetic peptide
LSESLKRIGDELDS

SEQ ID NO: 136 - protein, 13 aa, Artificial Sequence
  Description of Artificial Sequence: Synthetic peptide
CAVLLRLGDELEM

SEQ ID NO: 137 - protein, 10 aa, Artificial Sequence
  Description of Artificial Sequence: Synthetic peptide
  MOD_RES (1)..(1): Non-natural electrophile containing amino acid
XEVESATQLR

SEQ ID NO: 138 - protein, 6 aa, Artificial Sequence
  Description of Artificial Sequence: Synthetic peptide
  MOD_RES (1)..(1): Non-natural electrophile containing amino acid
XATQLR

SEQ ID NO: 139 - protein, 9 aa, Artificial Sequence
  Description of Artificial Sequence: Synthetic peptide
  MOD_RES (1)..(1): Non-natural electrophile containing amino acid
XVESATQLR

SEQ ID NO: 140 - protein, 8 aa, Artificial Sequence
  Description of Artificial Sequence: Synthetic peptide
  MOD_RES (1)..(1): Non-natural electrophile containing amino acid
XESATQLR

SEQ ID NO: 141 - protein, 7 aa, Artificial Sequence
  Description of Artificial Sequence: Synthetic peptide
  MOD_RES (1)..(1): Non-natural electrophile containing amino acid
XSATQLR

SEQ ID NO: 142 - protein, 5 aa, Artificial Sequence
  Description of Artificial Sequence: Synthetic peptide
  MOD_RES (5)..(5): Any cell permeability enhancing amino acid (e.g., amino acids that change or shift the distribution of charge or hydrophobic character) or a stability enhancing amino acid (e.g., non- native, D, or alpha methyl amino acid point mutations)
LNFRX

SEQ ID NO: 143 - protein, 6 aa, Artificial Sequence
  Description of Artificial Sequence: Synthetic peptide
  MOD_RES (6)..(6): Any cell permeability enhancing amino acid (e.g., amino acids that change or shift the distribution of charge or hydrophobic character) or a stability enhancing amino acid (e.g., non- native, D, or alpha methyl amino acid point mutations)
LNFRQX

SEQ ID NO: 144 - protein, 7 aa, Artificial Sequence
  Description of Artificial Sequence: Synthetic peptide
  MOD_RES (7)..(7): Any cell permeability enhancing amino acid (e.g., amino acids that change or shift the distribution of charge or hydrophobic character) or a stability enhancing amino acid (e.g., non- native, D, or alpha methyl amino acid point mutations)
LNFRQKX

SEQ ID NO: 145 - protein, 9 aa, Artificial Sequence
  Description of Artificial Sequence: Synthetic peptide
  MOD_RES (9)..(9): Any cell permeability enhancing amino acid (e.g., amino acids that change or shift the distribution of charge or hydrophobic character) or a stability enhancing amino acid (e.g., non- native, D, or alpha methyl amino acid point mutations)
LNFRQKLLX

SEQ ID NO: 146 - protein, 10 aa, Artificial Sequence
  Description of Artificial Sequence: Synthetic peptide
  MOD_RES (10)..(10): Any cell permeability enhancing amino acid (e.g., amino acids that change or shift the distribution of charge or hydrophobic character) or a stability enhancing amino acid (e.g., non- native, D, or alpha methyl amino acid point mutations)
LNFRQKLLKX

SEQ ID NO: 147 - protein, 7 aa, Artificial Sequence
  Description of Artificial Sequence: Synthetic peptide
  MOD_RES (1)..(1): Non-natural electrophile containing amino acid
XIAQELR

SEQ ID NO: 148 - protein, 6 aa, Artificial Sequence
  Description of Artificial Sequence: Synthetic peptide
  MOD_RES (1)..(1): Non-natural electrophile containing amino acid
XAQELR

SEQ ID NO: 149 - protein, 7 aa, Artificial Sequence
  Description of Artificial Sequence: Synthetic peptide
  MOD_RES (1)..(1): Non-natural electrophile containing amino acid
XAQELRR

SEQ ID NO: 150 - protein, 9 aa, Artificial Sequence
  Description of Artificial Sequence: Synthetic peptide
  MOD_RES (9)..(9): Any cell permeability enhancing amino acid (e.g., amino acids that change or shift the distribution of charge or hydrophobic character) or a stability enhancing amino acid (e.g., non- native, D, or alpha methyl amino acid point mutations)
FNAYYARKX

SEQ ID NO: 151 - protein, 9 aa, Artificial Sequence
  Description of Artificial Sequence: Synthetic peptide
  MOD_RES (9)..(9): Any cell permeability enhancing amino acid (e.g., amino acids that change or shift the distribution of charge or hydrophobic character) or a stability enhancing amino acid (e.g., non- native, D, or alpha methyl amino acid point mutations)
FNAYYARRX

SEQ ID NO: 152 - protein, 7 aa, Artificial Sequence
  Description of Artificial Sequence: Synthetic peptide
  MOD_RES (1)..(1): Non-natural electrophile containing amino acid
XLSESLK

SEQ ID NO: 153 - protein, 6 aa, Artificial Sequence
  Description of Artificial Sequence: Synthetic peptide
  MOD_RES (1)..(1): Non-natural electrophile containing amino acid
XSESLK

SEQ ID NO: 154 - protein, 6 aa, Artificial Sequence
  Description of Artificial Sequence: Synthetic peptide
  MOD_RES (6)..(6): Any cell permeability enhancing amino acid (e.g., amino acids that change or shift the distribution of charge or hydrophobic character) or a stability enhancing amino acid (e.g., non- native, D, or alpha methyl amino acid point mutations)
LDSNKX

SEQ ID NO: 155 - protein, 5 aa, Artificial Sequence
  Description of Artificial Sequence: Synthetic peptide
  MOD_RES (5)..(5): Any cell permeability enhancing amino acid (e.g., amino acids that change or shift the distribution of charge or hydrophobic character) or a stability enhancing amino acid (e.g., non- native, D, or alpha methyl amino acid point mutations)
LDSNX

SEQ ID NO: 156 - protein, 9 aa, Artificial Sequence
  Description of Artificial Sequence: Synthetic peptide
  MOD_RES (9)..(9): Any cell permeability enhancing amino acid (e.g., amino acids that change or shift the distribution of charge or hydrophobic character) or a stability enhancing amino acid (e.g., non- native, D, or alpha methyl amino acid point mutations)
IGDDINRRX

SEQ ID NO: 157 - protein, 8 aa, Artificial Sequence
  Description of Artificial Sequence: Synthetic peptide
  MOD_RES (8)..(8): Any cell permeability enhancing amino acid (e.g., amino acids that change or shift the distribution of charge or hydrophobic character) or a stability enhancing amino acid (e.g., non- native, D, or alpha methyl amino acid point mutations)
IGDDINRX

SEQ ID NO: 158 - protein, 15 aa, Artificial Sequence
  Description of Artificial Sequence: Synthetic peptide
  MOD_RES (1)..(1): Non-natural electrophile containing amino acid
XPGGRLAEVCTVLLR

SEQ ID NO: 159 - protein, 14 aa, Artificial Sequence
  Description of Artificial Sequence: Synthetic peptide
  MOD_RES (1)..(1): Non-natural electrophile containing amino acid
XGGRLAEVCTVLLR

SEQ ID NO: 160 - protein, 9 aa, Artificial Sequence
  Description of Artificial Sequence: Synthetic peptide
  MOD_RES (9)..(9): Any cell permeability enhancing amino acid (e.g., amino acids that change or shift the distribution of charge or hydrophobic character) or a stability enhancing amino acid (e.g., non- native, D, or alpha methyl amino acid point mutations)
ELEQIRPSX

SEQ ID NO: 161 - protein, 7 aa, Artificial Sequence
  Description of Artificial Sequence: Synthetic peptide
  MOD_RES (7)..(7): Any cell permeability enhancing amino acid (e.g., amino acids that change or shift the distribution of charge or hydrophobic character) or a stability enhancing amino acid (e.g., non- native, D, or alpha methyl amino acid point mutations)
ELEQIRX

SEQ ID NO: 162 - protein, 12 aa, Artificial Sequence
  Description of Artificial Sequence: Synthetic peptide
  MOD_RES (1)..(1): Non-natural electrophile containing amino acid
XDIIRNIARHLA

SEQ ID NO: 163 - protein, 11 aa, Artificial Sequence
  Description of Artificial Sequence: Synthetic peptide
  MOD_RES (1)..(1): Non-natural electrophile containing amino acid
XIIRNIARHLA

SEQ ID NO: 164 - protein, 6 aa, Artificial Sequence
  Description of Artificial Sequence: Synthetic peptide
  MOD_RES (1)..(1): Norleucine
  MOD_RES (6)..(6): Any cell permeability enhancing amino acid (e.g., amino acids that change or shift the distribution of charge or hydrophobic character) or a stability enhancing amino acid (e.g., non- native, D, or alpha methyl amino acid point mutations)
XDRSIX

SEQ ID NO: 165 - protein, 7 aa, Artificial Sequence
  Description of Artificial Sequence: Synthetic peptide
  MOD_RES (1)..(1): Norleucine
  MOD_RES (7)..(7): Any cell permeability enhancing amino acid (e.g., amino acids that change or shift the distribution of charge or hydrophobic character) or a stability enhancing amino acid (e.g., non- native, D, or alpha methyl amino acid point mutations)
XDRSIRX

SEQ ID NO: 166 - protein, 13 aa, Artificial Sequence
  Description of Artificial Sequence: Synthetic peptide
  MOD_RES (1)..(1): Non-natural electrophile containing amino acid
XEQWAREIGAQLR

SEQ ID NO: 167 - protein, 12 aa, Artificial Sequence
  Description of Artificial Sequence: Synthetic peptide
  MOD_RES (1)..(1): Non-natural electrophile containing amino acid
XQWAREIGAQLR

SEQ ID NO: 168 - protein, 9 aa, Artificial Sequence
  Description of Artificial Sequence: Synthetic peptide
  MOD_RES (1)..(1): Non-natural electrophile containing amino acid
XREIGAQLR

SEQ ID NO: 169 - protein, 8 aa, Artificial Sequence
  Description of Artificial Sequence: Synthetic peptide
  MOD_RES (1)..(1): Non-natural electrophile containing amino acid
XEIGAQLR

SEQ ID NO: 170 - protein, 6 aa, Artificial Sequence
  Description of Artificial Sequence: Synthetic peptide
  MOD_RES (6)..(6): Any cell permeability enhancing amino acid (e.g., amino acids that change or shift the distribution of charge or hydrophobic character) or a stability enhancing amino acid (e.g., non- native, D, or alpha methyl amino acid point mutations)
LNAQYX

SEQ ID NO: 171 - protein, 7 aa, Artificial Sequence
  Description of Artificial Sequence: Synthetic peptide
  MOD_RES (7)..(7): Any cell permeability enhancing amino acid (e.g., amino acids that change or shift the distribution of charge or hydrophobic character) or a stability enhancing amino acid (e.g., non- native, D, or alpha methyl amino acid point mutations)
LNAQYEX

SEQ ID NO: 172 - protein, 8 aa, Artificial Sequence
  Description of Artificial Sequence: Synthetic peptide
  MOD_RES (8)..(8): Any cell permeability enhancing amino acid (e.g., amino acids that change or shift the distribution of charge or hydrophobic character) or a stability enhancing amino acid (e.g., non- native, D, or alpha methyl amino acid point mutations)
LNFRQKLX

SEQ ID NO: 173 - protein, 25 aa, Artificial Sequence
  Description of Artificial Sequence: Synthetic peptide
  MOD_RES (1)..(1): Non-natural electrophile containing amino acid
  MISC_FEATURE (2)..(5): May or may not be present
  MISC_FEATURE (2)..(10): This region may encompass "EVESATQLR" or "VESATQLR" or "ESATQLR" or "SATQLR" or "ATQLR" wherein some positions may be absent
  MOD_RES (11)..(11): Any amino acid
  MOD_RES (15)..(15): Any amino acid
  MISC_FEATURE (16)..(24): This region may encompass "LNFRQKLLK" or "LNFRQKLL" or "LNFRQKL" or "LNFRQK" or "LNFRQ" or "LNFR" wherein some positions may be absent
  MISC_FEATURE (20)..(24): May or may not be present
  MOD_RES (25)..(25): Any cell permeability enhancing amino acid (e.g., amino acids that change or shift the distribution of charge or hydrophobic character) or a stability enhancing amino acid (e.g., non- native, D, or alpha methyl amino acid point mutations)
  See specification as filed for detailed description of substitutions and preferred embodiments
XEVESATQLRXFGDXLNFRQKLLKX

SEQ ID NO: 174 - protein, 22 aa, Artificial Sequence
  Description of Artificial Sequence: Synthetic peptide
  MOD_RES (1)..(1): Non-natural electrophile containing amino acid
  MISC_FEATURE (2)..(2): May or may not be present
  MISC_FEATURE (2)..(8): This region may encompass "IAQELR" or "AQELR" or "AQELRR" wherein some positions may be absent
  MISC_FEATURE (8)..(8): May or may not be present
  MOD_RES (9)..(9): Any amino acid
  MOD_RES (13)..(13): Any amino acid
  MISC_FEATURE (14)..(21): This region may encompass "FNAYYARK" or "FNAYYARR" wherein some positions may be absent
  MOD_RES (21)..(21): Arg or Lys
  MOD_RES (22)..(22): Any cell permeability enhancing amino acid (e.g., amino acids that change or shift the distribution of charge or hydrophobic character) or a stability enhancing amino acid (e.g., non- native, D, or alpha methyl amino acid point mutations)
  See specification as filed for detailed description of substitutions and preferred embodiments
XIAQELRRXIGDXFNAYYARXX

SEQ ID NO: 175 - protein, 18 aa, Artificial Sequence
  Description of Artificial Sequence: Synthetic peptide
  MOD_RES (1)..(1): Non-natural electrophile containing amino acid
  MISC_FEATURE (2)..(2): May or may not be present
  MISC_FEATURE (2)..(7): This region may encompass "LSESLK" or "SESLK" wherein some positions may be absent
  MOD_RES (8)..(8): Any amino acid
  MOD_RES (12)..(12): Any amino acid
  MISC_FEATURE (13)..(17): This region may encompass "LDSNK" or "LDSN" wherein some positions may be absent
  MISC_FEATURE (17)..(17): May or may not be present
  MOD_RES (18)..(18): Any cell permeability enhancing amino acid (e.g., amino acids that change or shift the distribution of charge or hydrophobic character) or a stability enhancing amino acid (e.g., non- native, D, or alpha methyl amino acid point mutations)
  See specification as filed for detailed description of substitutions and preferred embodiments
XLSESLKXIGDXLDSNKX

SEQ ID NO: 176 - protein, 17 aa, Artificial Sequence
  Description of Artificial Sequence: Synthetic peptide
  MOD_RES (1)..(1): Non-natural electrophile containing amino acid
  MISC_FEATURE (2)..(2): May or may not be present
  MISC_FEATURE (2)..(3): This region may encompass "VG" or "G" wherein some positions may be absent
  MOD_RES (4)..(4): Any amino acid
  MOD_RES (8)..(8): Any amino acid
  MISC_FEATURE (9)..(16): This region may encompass "IGDDINRR" or "IGDDINR" wherein some positions may be absent
  MISC_FEATURE (16)..(16): May or may not be present
  MOD_RES (17)..(17): Any cell permeability enhancing amino acid (e.g., amino acids that change or shift the distribution of charge or hydrophobic character) or a stability enhancing amino acid (e.g., non- native, D, or alpha methyl amino acid point mutations)
  See specification as filed for detailed description of substitutions and preferred embodiments
XVGXQLAXIGDDINRRX

SEQ ID NO: 177 - protein, 29 aa, Artificial Sequence
  Description of Artificial Sequence: Synthetic peptide
  MOD_RES (1)..(1): Non-natural electrophile containing amino acid
  MISC_FEATURE (2)..(2): May or may not be present
  MISC_FEATURE (2)..(15): This region may encompass "PGGRLAEVCTVLLR" or "GGRLAEVCTVLLR" wherein some positions may be absent
  MOD_RES (16)..(16): Any amino acid
  MOD_RES (20)..(20): Any amino acid
  MISC_FEATURE (21)..(28): This region may encompass "ELEQIRPS" or "ELEQIR" wherein some positions may be absent
  MISC_FEATURE (27)..(28): May or may not be present
  MOD_RES (29)..(29): Any cell permeability enhancing amino acid (e.g., amino acids that change or shift the distribution of charge or hydrophobic character) or a stability enhancing amino acid (e.g., non- native, D, or alpha methyl amino acid point mutations)
  See specification as filed for detailed description of substitutions and preferred embodiments
XPGGRLAEVCTVLLRXLGDXELEQIRPSX

SEQ ID NO: 178 - protein, 24 aa, Artificial Sequence
  Description of Artificial Sequence: Synthetic peptide
  MOD_RES (1)..(1): Non-natural electrophile containing amino acid
  MISC_FEATURE (2)..(2): May or may not be present
  MISC_FEATURE (2)..(12): This region may encompass "DIIRNIARHLA" or "IIRNIARHLA" wherein some positions may be absent
  MOD_RES (13)..(13): Any amino acid
  MOD_RES (17)..(17): Any amino acid
  MOD_RES (18)..(18): Norleucine
  MISC_FEATURE (18)..(23): This region may encompass "BDRSIR" or "BDRSI" wherein B is norleucine and some positions may be absent
  MISC_FEATURE (23)..(23): May or may not be present
  MOD_RES (24)..(24): Any cell permeability enhancing amino acid (e.g., amino acids that change or shift the distribution of charge or hydrophobic character) or a stability enhancing amino acid (e.g., non- native, D, or alpha methyl amino acid point mutations)
  See specification as filed for detailed description of substitutions and preferred embodiments
XDIIRNIARHLAXVGDXXDRSIRX

SEQ ID NO: 179 - protein, 25 aa, Artificial Sequence
  Description of Artificial Sequence: Synthetic peptide
  MOD_RES (1)..(1): Non-natural electrophile containing amino acid
  MISC_FEATURE (2)..(6): May or may not be present
  MISC_FEATURE (2)..(13): This region may encompass "EQWAREIGAQLR" or "QWAREIGAQLR" "REIGAQLR" or "EIGAQLR" wherein some positions may be absent
  MOD_RES (14)..(14): Any amino acid
  MOD_RES (15)..(15): Met or norleucine
  MOD_RES (18)..(18): Any amino acid
  MISC_FEATURE (19)..(24): This region may encompass "LNAQYE" or "LNAQY" wherein some positions may be absent
  MISC_FEATURE (24)..(24): May or may not be present
  MOD_RES (25)..(25): Any cell permeability enhancing amino acid (e.g., amino acids that change or shift the distribution of charge or hydrophobic character) or a stability enhancing amino acid (e.g., non- native, D, or alpha methyl amino acid point mutations)
  See specification as filed for detailed description of substitutions and preferred embodiments
XEQWAREIGAQLRXXADXLNAQYEX

SEQ ID NO: 180 - protein, 26 aa, Artificial Sequence
  Description of Artificial Sequence: Synthetic peptide
  MOD_RES (1)..(1): beta-Ala
  MOD_RES (14)..(14): Any non-natural amino acid
  MOD_RES (18)..(18): Any non-natural amino acid
AAELEVECATQLRXFGDXLNFRQKLL

SEQ ID NO: 181 - protein, 26 aa, Artificial Sequence
  Description of Artificial Sequence: Synthetic peptide
  MOD_RES (1)..(1): beta-Ala
  MOD_RES (14)..(14): Any non-natural amino acid
  MOD_RES (18)..(18): Any non-natural amino acid
AAELEVECATQLRXFGDXLNFRQKLL

SEQ ID NO: 182 - protein, 26 aa, Artificial Sequence
  Description of Artificial Sequence: Synthetic peptide
  MOD_RES (1)..(1): beta-Ala
  MOD_RES (14)..(14): Any non-natural amino acid
  MOD_RES (18)..(18): Any non-natural amino acid
AAELEVESATQLRXFGDXLNFRQKLL

SEQ ID NO: 183 - protein, 26 aa, Artificial Sequence
  Description of Artificial Sequence: Synthetic peptide
  MOD_RES (1)..(1): beta-Ala
  MOD_RES (14)..(14): Any non-natural amino acid
  MOD_RES (18)..(18): Any non-natural amino acid
AAELEVESATQLRXFGDXLNFRQKLL

SEQ ID NO: 184 - protein, 23 aa, Artificial Sequence
  Description of Artificial Sequence: Synthetic peptide
  MOD_RES (10)..(10): Any non-natural amino acid
  MOD_RES (14)..(14): Any non-natural amino acid
EVESATQLRXFGDXLNFRQKLLK

SEQ ID NO: 185 - protein, 23 aa, Artificial Sequence
  Description of Artificial Sequence: Synthetic peptide
  MOD_RES (10)..(10): Any non-natural amino acid
  MOD_RES (14)..(14): Any non-natural amino acid
EVESATQLRXFGDXLNFRQKLLK

SEQ ID NO: 186 - protein, 22 aa, Artificial Sequence
  Description of Artificial Sequence: Synthetic peptide
  MOD_RES (10)..(10): Any non-natural amino acid
  MOD_RES (14)..(14): Any non-natural amino acid
EVESATQLRXFGDXLNFRQKLL

SEQ ID NO: 187 - protein, 23 aa, Artificial Sequence
  Description of Artificial Sequence: Synthetic peptide
  MOD_RES (10)..(10): Any non-natural amino acid
  MOD_RES (14)..(14): Any non-natural amino acid
EVESATQLRXFGDXLNFRQKLLK

SEQ ID NO: 188 - protein, 23 aa, Artificial Sequence
  Description of Artificial Sequence: Synthetic peptide
  MOD_RES (10)..(10): Any non-natural amino acid
  MOD_RES (14)..(14): Any non-natural amino acid
EVESATQLRXFGDXLNFRQKLLK

SEQ ID NO: 189 - protein, 23 aa, Artificial Sequence
  Description of Artificial Sequence: Synthetic peptide
  MOD_RES (10)..(10): Any non-natural amino acid
  MOD_RES (14)..(14): Any non-natural amino acid
EVESATQLRXFGDXLNFRQKLLK

SEQ ID NO: 190 - protein, 23 aa, Artificial Sequence
  Description of Artificial Sequence: Synthetic peptide
  MOD_RES (10)..(10): Any non-natural amino acid
  MOD_RES (14)..(14): Any non-natural amino acid
EVESATQLRXFGDXLNFRQKLLK

SEQ ID NO: 191 - protein, 23 aa, Artificial Sequence
  Description of Artificial Sequence: Synthetic peptide
  MOD_RES (10)..(10): Any non-natural amino acid
  MOD_RES (14)..(14): Any non-natural amino acid
EVESATQLRXFGDXLNFRQKLLK

SEQ ID NO: 192 - protein, 23 aa, Artificial Sequence
  Description of Artificial Sequence: Synthetic peptide
  MOD_RES (10)..(10): Any non-natural amino acid
  MOD_RES (14)..(14): Any non-natural amino acid
EVESATQLRXFGDXLNFRQKLLK

SEQ ID NO: 193 - protein, 22 aa, Artificial Sequence
  Description of Artificial Sequence: Synthetic peptide
  MOD_RES (10)..(10): Any non-natural amino acid
  MOD_RES (14)..(14): Any non-natural amino acid
EVESATQLRXFGDXLNFRQKLL

SEQ ID NO: 194 - protein, 23 aa, Artificial Sequence
  Description of Artificial Sequence: Synthetic peptide
  MOD_RES (10)..(10): Any non-natural amino acid
  MOD_RES (14)..(14): Any non-natural amino acid
EVESATQLRXFGDXLNFRQKLLK

SEQ ID NO: 195 - protein, 19 aa, Artificial Sequence
  Description of Artificial Sequence: Synthetic peptide
  MOD_RES (7)..(7): Any non-natural amino acid
  MOD_RES (11)..(11): Any non-natural amino acid
IAQELRXIGDXFNAYYARK

SEQ ID NO: 196 - protein, 19 aa, Artificial Sequence
  Description of Artificial Sequence: Synthetic peptide
  MOD_RES (7)..(7): Any non-natural amino acid
  MOD_RES (11)..(11): Any non-natural amino acid
IAQELRXIGDXFNAYYARK

SEQ ID NO: 197 - protein, 19 aa, Artificial Sequence
  Description of Artificial Sequence: Synthetic peptide
  MOD_RES (7)..(7): Any non-natural amino acid
  MOD_RES (11)..(11): Any non-natural amino acid
IAQELRXIGDXFNAYYARR

SEQ ID NO: 198 - protein, 20 aa, Artificial Sequence
  Description of Artificial Sequence: Synthetic peptide
  MOD_RES (7)..(7): Any non-natural amino acid
  MOD_RES (11)..(11): Any non-natural amino acid
IAQELRXIGDXFNAYYARRK

SEQ ID NO: 199 - protein, 19 aa, Artificial Sequence
  Description of Artificial Sequence: Synthetic peptide
  MOD_RES (7)..(7): Any non-natural amino acid
  MOD_RES (11)..(11): Any non-natural amino acid
IAQELRXIGDXFNAYYARK

SEQ ID NO: 200 - protein, 19 aa, Artificial Sequence
  Description of Artificial Sequence: Synthetic peptide
  MOD_RES (7)..(7): Any non-natural amino acid
  MOD_RES (11)..(11): Any non-natural amino acid
IAQELRXIGDXFNAYYARK

SEQ ID NO: 201 - protein, 19 aa, Artificial Sequence
  Description of Artificial Sequence: Synthetic peptide
  MOD_RES (7)..(7): Any non-natural amino acid
  MOD_RES (11)..(11): Any non-natural amino acid
IAQELRXIGDXFNAYYARK

SEQ ID NO: 202 - protein, 19 aa, Artificial Sequence
  Description of Artificial Sequence: Synthetic peptide
  MOD_RES (7)..(7): Any non-natural amino acid
  MOD_RES (11)..(11): Any non-natural amino acid
IAQELRXIGDXFNAYYARK

SEQ ID NO: 203 - protein, 19 aa, Artificial Sequence
  Description of Artificial Sequence: Synthetic peptide
  MOD_RES (7)..(7): Any non-natural amino acid
  MOD_RES (11)..(11): Any non-natural amino acid
IAQELRXIGDXFANYYARK

SEQ ID NO: 204 - protein, 19 aa, Artificial Sequence
  Description of Artificial Sequence: Synthetic peptide
  MOD_RES (7)..(7): Any non-natural amino acid
  MOD_RES (11)..(11): Any non-natural amino acid
IAQELRXIGDXFNAYYARR

SEQ ID NO: 205 - protein, 20 aa, Artificial Sequence
  Description of Artificial Sequence: Synthetic peptide
  MOD_RES (7)..(7): Any non-natural amino acid
  MOD_RES (11)..(11): Any non-natural amino acid
IAQELRXIGDXFNAYYARRK

SEQ ID NO: 206 - protein, 22 aa, Artificial Sequence
  Description of Artificial Sequence: Synthetic peptide
  MOD_RES (1)..(1): beta-Ala
  MOD_RES (10)..(10): Any non-natural amino acid
  MOD_RES (14)..(14): Any non-natural amino acid
AIWIAQELRXIGDXFNAYYARR

SEQ ID NO: 207 - protein, 19 aa, Artificial Sequence
  Description of Artificial Sequence: Synthetic peptide
  MOD_RES (7)..(7): Any non-natural amino acid
  MOD_RES (11)..(11): Any non-natural amino acid
IAQELRXIGDXFNAYYARR

SEQ ID NO: 208 - protein, 21 aa, Artificial Sequence
  Description of Artificial Sequence: Synthetic peptide
  MOD_RES (9)..(9): Any non-natural amino acid
  MOD_RES (13)..(13): Any non-natural amino acid
IWIAQELRXIGDXFNAYYARR

SEQ ID NO: 209 - protein, 25 aa, Artificial Sequence
  Description of Artificial Sequence: Synthetic peptide
AELEVECATQLRRFGDKLNFRQKLL

SEQ ID NO: 210 - protein, 9 aa, Artificial Sequence
  Description of Artificial Sequence: Synthetic 9xHis tag
HHHHHHHHH